European Patent Specification EP 3 856 921 B1, published April 29, 2026. Title: LUNG PROTEASE NANOSENSORS AND USES THEREOF. Applicant: MASSACHUSETTS INSTITUTE OF TECHNOLOGY. Application Not Yet Assigned. The sequence listing filed with the application follows.

SEQUENCE LISTING (48 sequences)

SEQ ID NO: 1 - protein, 7 aa, Artificial Sequence
  Synthetic Polypeptide
PQGIWGQ

SEQ ID NO: 2 - protein, 6 aa, Artificial Sequence
  Synthetic Polypeptide
PVGLIG

SEQ ID NO: 3 - protein, 8 aa, Artificial Sequence
  Synthetic Polypeptide
PVPLSLVM

SEQ ID NO: 4 - protein, 7 aa, Artificial Sequence
  Synthetic Polypeptide
PLGLRSW

SEQ ID NO: 5 - protein, 7 aa, Artificial Sequence
  Synthetic Polypeptide
PLGVRGK

SEQ ID NO: 6 - protein, 7 aa, Artificial Sequence
  Synthetic Polypeptide
  MISC_FEATURE (1)..(1): d-Phe
FPRSGGG

SEQ ID NO: 7 - protein, 8 aa, Artificial Sequence
  Synthetic Polypeptide
LGPKGQTG

SEQ ID NO: 8 - protein, 10 aa, Artificial Sequence
  Synthetic Polypeptide
GSGRSANAKG

SEQ ID NO: 9 - protein, 9 aa, Artificial Sequence
  Synthetic Polypeptide
KPISLISSG

SEQ ID NO: 10 - protein, 9 aa, Artificial Sequence
  Synthetic Polypeptide
ILSRIVGGG

SEQ ID NO: 11 - protein, 9 aa, Artificial Sequence
  Synthetic Polypeptide
SGSKIIGGG

SEQ ID NO: 12 - protein, 7 aa, Artificial Sequence
  Synthetic Polypeptide
PLGMRGG

SEQ ID NO: 13 - protein, 7 aa, Artificial Sequence
  Synthetic Polypeptide
  MISC_FEATURE (2)..(2): Xaa is 3-cyclohexylalanine
  MISC_FEATURE (4)..(4): Methyl-cysteine
PXGCHAG

SEQ ID NO: 14 - protein, 8 aa, Artificial Sequence
  Synthetic Polypeptide
APFEMSAG

SEQ ID NO: 15 - protein, 14 aa, Artificial Sequence [sequence omitted]

SEQ ID NO: 16 - protein, 14 aa, Artificial Sequence [sequence omitted]

SEQ ID NO: 17 - protein, 14 aa, Artificial Sequence [sequence omitted]

SEQ ID NO: 18 - protein, 14 aa, Artificial Sequence [sequence omitted]

SEQ ID NO: 19 - protein, 14 aa, Artificial Sequence [sequence omitted]

SEQ ID NO: 20 - protein, 14 aa, Artificial Sequence [sequence omitted]

SEQ ID NO: 21 - protein, 14 aa, Artificial Sequence [sequence omitted]

SEQ ID NO: 22 - protein, 14 aa, Artificial Sequence [sequence omitted]

SEQ ID NO: 23 - protein, 14 aa, Artificial Sequence [sequence omitted]

SEQ ID NO: 24 - protein, 14 aa, Artificial Sequence [sequence omitted]

SEQ ID NO: 25 - protein, 14 aa, Artificial Sequence [sequence omitted]

SEQ ID NO: 26 - protein, 14 aa, Artificial Sequence [sequence omitted]

SEQ ID NO: 27 - protein, 14 aa, Artificial Sequence [sequence omitted]

SEQ ID NO: 28 - protein, 14 aa, Artificial Sequence [sequence omitted]

SEQ ID NO: 29 - protein, 11 aa, Artificial Sequence
  Synthetic Polypeptide
  MISC_FEATURE (10)..(10): modified by CPQ2-PEG2
GGPQGIWGQKC

SEQ ID NO: 30 - protein, 10 aa, Artificial Sequence
  Synthetic Polypeptide
  MISC_FEATURE (9)..(9): modified by CPQ2-PEG2
GGPVGLIGKC

SEQ ID NO: 31 - protein, 12 aa, Artificial Sequence
  Synthetic Polypeptide
  MISC_FEATURE (11)..(11): modified by CPQ2-PEG2
GGPVPLSLVMKC

SEQ ID NO: 32 - protein, 11 aa, Artificial Sequence
  Synthetic Polypeptide
  MISC_FEATURE (10)..(10): modified by CPQ2-PEG2
GGPLGLRSWKC

SEQ ID NO: 33 - protein, 11 aa, Artificial Sequence
  Synthetic Polypeptide
  MISC_FEATURE (10)..(10): modified by CPQ2-PEG2
GGPLGVRGKKC

SEQ ID NO: 34 - protein, 11 aa, Artificial Sequence
  Synthetic Polypeptide
  MISC_FEATURE (3)..(3): d-Phe
  MISC_FEATURE (10)..(10): modified by CPQ2-PEG2
GGFPRSGGGKC

SEQ ID NO: 35 - protein, 14 aa, Artificial Sequence
  Synthetic Polypeptide
  MISC_FEATURE (11)..(11): modified by CPQ2
  MISC_FEATURE (12)..(13): d-Lys
  MISC_FEATURE (13)..(13): modified by PEG2
GGLGPKGQTGKKKC

SEQ ID NO: 36 - protein, 15 aa, Artificial Sequence
  Synthetic Polypeptide
  MISC_FEATURE (13)..(13): modified by CPQ2-PEG2
GGGSGRSANAKGKGC

SEQ ID NO: 37 - protein, 13 aa, Artificial Sequence
  Synthetic Polypeptide
  MISC_FEATURE (11)..(11): modified by CPQ2-PEG2
GKPISLISSGKGC

SEQ ID NO: 38 - protein, 13 aa, Artificial Sequence
  Synthetic Polypeptide
  MISC_FEATURE (11)..(11): modified by CPQ2-PEG2
GILSRIVGGGKGC

SEQ ID NO: 39 - protein, 13 aa, Artificial Sequence
  Synthetic Polypeptide
  MISC_FEATURE (11)..(11): modified by CPQ2-PEG2
GSGSKIIGGGKGC

SEQ ID NO: 40 - protein, 12 aa, Artificial Sequence
  Synthetic Polypeptide
  MISC_FEATURE (10)..(10): modified by CPQ2
GGPLGMRGGKGC

SEQ ID NO: 41 - protein, 11 aa, Artificial Sequence
  Synthetic Polypeptide
  MISC_FEATURE (3)..(3): Xaa is 3-cyclohexylalanine
  MISC_FEATURE (5)..(5): methyl-cysteine
  MISC_FEATURE (9)..(9): modified by CPQ2
GPXGCHAGKGC

SEQ ID NO: 42 - protein, 12 aa, Artificial Sequence
  Synthetic Polypeptide
  MISC_FEATURE (10)..(10): modified by CPQ2
GAPFEMSAGKGC

SEQ ID NO: 43 - protein, 5 aa, Artificial Sequence
  Synthetic Polypeptide
LGGGA

SEQ ID NO: 44 - protein, 4 aa, Artificial Sequence
  Synthetic Polypeptide
AAFA

SEQ ID NO: 45 - protein, 8 aa, Artificial Sequence
  Synthetic Polypeptide
  MISC_FEATURE (8)..(8): modified by FAM
GLGGGAGK

SEQ ID NO: 46 - protein, 23 aa, Artificial Sequence
  Synthetic Polypeptide
  MISC_FEATURE (1)..(1): d-Glu
  MISC_FEATURE (3)..(3): d-Val
  MISC_FEATURE (4)..(4): d-Asn
  MISC_FEATURE (5)..(5): d-Asp
  MISC_FEATURE (6)..(7): d-Glu
  MISC_FEATURE (9)..(10): d-Phe
  MISC_FEATURE (11)..(11): d-Ser
  MISC_FEATURE (12)..(12): d-Ala
  MISC_FEATURE (13)..(13): d-Arg
  MISC_FEATURE (14)..(14): modified by AF488
EGVNDEEGFFSARKGGLGGGAGC

SEQ ID NO: 47 - protein, 7 aa, Artificial Sequence
  Synthetic Polypeptide
  MISC_FEATURE (7)..(7): modified by FAM
GAAFAGK

SEQ ID NO: 48 - protein, 22 aa, Artificial Sequence
  Synthetic Polypeptide
  MISC_FEATURE (1)..(1): d-Glu
  MISC_FEATURE (3)..(3): d-Val
  MISC_FEATURE (4)..(4): d-Asn
  MISC_FEATURE (5)..(5): d-Asp
  MISC_FEATURE (6)..(7): d-Glu
  MISC_FEATURE (9)..(10): d-Phe
  MISC_FEATURE (11)..(11): d-Ser
  MISC_FEATURE (12)..(12): d-Ala
  MISC_FEATURE (13)..(13): d-Arg
  MISC_FEATURE (14)..(14): modified by FAM
EGVNDEEGFFSARKGGAAFAGC